European Patent Specification EP 3 273 989 B1, published December 27, 2023. Title: Streptococcal Vaccine. Applicant: Gamma Vaccines Pty Limited. The sequence listing filed with the application follows.

SEQUENCE LISTING (6 sequences)

SEQ ID NO: 1 - DNA, 1324 bp, Streptococcus pneumoniae
tgaaaatagtttaacagacttttgacttcttttatatgatataataaagtatagtatttatgaaaaggacatatagagactgtaaaaatatacttttgaaaatctttttagtctggggtgttattgtagatagaatgcagaccttgtcagtcctatttacagtgtcaaaatagtgcgttttgaagttctatctacaagcctaatcgtgactaagattgtcttctttgtaaggtagaaataaaggagtttctggttctggattgtaaaaaatgagttgttttaattgataaggagtagaatatggaaattaatgtgagtaaattaagaacagatttgcctcaagtcggcgtgcaaccatataggcaagtacacgcacactcaactgggaatccgcattcaaccgtacagaatgaagcggattatcactggcggaaagacccagaattaggttttttctcgcacattgttgggaacggttgcatcatgcaggtaggacctgttgataatggtgcctgggacgttgggggcggttggaatgctgagacctatgcagcggttgaactgattgaaagccattcaaccaaagaagagttcatgacggactaccgcctttatatcgaactcttacgcaatctagcagatgaagcaggtttgccgaaaacgcttgatacagggagtttagctggaattaaaacgcacgagtattgcacgaataaccaaccaaacaaccactcagaccacgttgacccttatccatatcttgctaaatggggcattagccgtgagcagtttaagcatgatattgagaacggcttgacgattgaaacaggctggcagaagaatgacactggctactggtacgtacattcagacggctcttatccaaaagacaagtttgagaaaatcaatggcacttggtactactttgacagttcaggctatatgcttgcagaccgctggaggaagcacacagacggcaactggtactggttcgacaactcaggcgaaatggctacaggctggaagaaaatcgctgataagtggtactatttcaacgaagaaggtgccatgaagacaggctgggtcaagtacaaggacacttggtactacttagacgctaaagaaggcgccatggtatcaaatgcctttatccagtcagcggacggaacaggctggtactacctcaaaccagacggaacactggcagacaagccagaattcacagtagagccagatggcttgattacagtaaaataataatggaatgtctttcaaatcagaacagcgcatattattaggtcttgaaaaagcttaatagtatgcg

SEQ ID NO: 2 - DNA, 367 bp, Streptococcus pneumoniae
tgaaaatagtttaacagacttttgacttcttttatatgatataataaagtatagtatttatgaaaaggacatatagagactgtaaaaatatacttttgaaaatctttttagtctggggtgttattgtagatagaatgcagaccttgtcagtcctatttacagtgtcaaaatagtgcgttttgaagttctatctacaagcctaatcgtgactaagattgtcttctttgtaaggtagaaataaaggagtttctggttctggattgtaaaaaatgagttgttttaattgataaggagtagaattaatggaatgtctttcaaatcagaacagcgcatattattaggtcttgaaaaagcttaatagtatgcg

SEQ ID NO: 3 - RNA, 234 nt, Streptococcus pneumoniae
aaugcagaccuugucaguccuauuuacagugucaaaauagugcguuuugaaguucuaucuacaagccuaaucgugacuaagauugucuucuuuguaagguagaaauaaaggaguuucugguucuggauuguaaaaaaugaguuguuuuaauugauaaggaguagaauuaauggaaugucuuucaaaucagaacagcgcauauuauuaggucuugaaaaagcuuaauaguaugcg

SEQ ID NO: 4 - DNA, 1140 bp, Streptococcus pneumoniae
cagttttgggactctttattggctatagttttaatgttgcggcaggttctagtatcgtgcttacagctgctagtttctttctcattagcttctttatcgctcccaaacaacgatatttgaaactgaaaaataaacatttgttaaaataaggggcaaagccctaataaattggaggatctaatgaaaaaattaggtacattactcgttctctttctttctgcaatcattcttgtagcatgtgctagcggaaaaaaagatacaacttctggtcaaaaactaaaagttgttgctacaaactcaatcatcgctgatattactaaaaatattgctggtgacaaaattgaccttcatagtatcgttccgattgggcaagacccacacgaatacgaaccacttcctgaagacgttaagaaaacttctgaggctgatttgattttctataacggtatcaaccttgaaacaggtggcaatgcttggtttacaaaattggtagaaaatgccaagaaaactgaaaacaaagactacttcgcagtcagcgacggcgttgatgttatctaccttgaaggtcaaaatgaaaaaggaaaagaagacccacacgcttggcttaaccttgaaaacggtattatttttgctaaaaatatcgccaaacaattgagcgccaaagaccctaacaataaagaattctatgaaaaaaatctcaaagaatatactgataagttagacaaacttgataaagaaagtaaggataaatttaataagatccctgctgaaaagaaactcattgtaaccagcgaaggagcattcaaatacttctctaaagcctatggtgttccaagtgcctacatctgggaaatcaatactgaagaagaaggaactcctgaacaaatcaagaccttggttgaaaaacttcgccaaacaaaagttccatcactctttgtagaatcaagtgtggatgaccgtccaatgaaaactgtttctcaagacacaaacatcccaatctacgcacaaatctttactgactctatcgcagaacaaggtaaagaaggcgacagctactacagcatgatgaaatacaaccttgacaagattgctgaaggattggcaaaataagcctctgaaaaacgtcattctcatgtgagc

SEQ ID NO: 5 - DNA, 281 bp, Streptococcus pneumoniae
cagttttgggactctttattggctatagttttaatgttgcggcaggttctagtatcgtgcttacagctgctagtttctttctcattagcttctttatcgctcccaaacaacgatatttgaaactgaaaaataaacatttgttaaaataaggggcaaagccctaataaattgggtaaagaaggcgacagctactacagcatgatgaaatacaaccttgacaagattgctgaaggattggcaaaataagcctctgaaaaacgtcattctcatgtgagctggcg

SEQ ID NO: 6 - RNA, 110 nt, Streptococcus pneumoniae
gguaaagaaggcgacagcuacuacagcaugaugaaauacaaccuugacaagauugcugaaggauuggcaaaauaagccucugaaaaacgucauucucaugugagcuggcg